European Patent Specification EP 3 830 284 B1, published February 19, 2025. Title: Bacterial Vaginosis Diagnostic. Applicant: Mologic Ltd. The sequence listing filed with the application follows.

SEQUENCE LISTING (17 sequences)

SEQ ID NO: 1 - protein, 7 aa, Oryctolagus cuniculus
GFSLSSY

SEQ ID NO: 2 - protein, 5 aa, Oryctolagus cuniculus
TTTLH

SEQ ID NO: 3 - protein, 6 aa, Oryctolagus cuniculus
GGSSVI

SEQ ID NO: 4 - protein, 13 aa, Oryctolagus cuniculus
QSSQSVYGNNHLN

SEQ ID NO: 5 - protein, 7 aa, Oryctolagus cuniculus
SASRLAS

SEQ ID NO: 6 - protein, 12 aa, Oryctolagus cuniculus
QGSYYNGAWYVA

SEQ ID NO: 7 - protein, 434 aa, Oryctolagus cuniculus
QSVEESGGRLVTPGTPLTLTCTVSGFSLSSYSMDWVRQAPGKGLEWVGGITTTLHTFYATWAKGRFTISKTSSTTVDLKMTSLTTDDAATYFCARGGSSVIWGPGTLVTVSSGQPKAPSVFPLAPCCGDTPSSTVTLGCLVKGYLPEPVTVTWNSGTLTNGVRTFPSVRQSSGLYSLSSVVSVTSSSQPVTCNVAHPATNTKVDKTVAPSTCSKPTCPPPELLGGPSVFIFPPKPKDTLMISRTPEVTCVVVDVSEDDPEVQFTWYINNEQVRTARPPLREQQFNSTIRVVSTLPIAHEDWLRGKEFKCKVHNKALPAPIEKTISKARGQPLEPKVYTMGPPREELSSRSVSLTCMINGFYPSDISVEWEKNGKAEDNYKTTPAVLDSDGSYFLYSKLSVPTSEWQRGDVFTCSVMHEALHNHYTQKSISRSPG

SEQ ID NO: 8 - protein, 218 aa, Oryctolagus cuniculus
ALVMTQTPSPVSAAVGGTVTISCQSSQSVYGNNHLNWHQQKRGQPPKQLIGSASRLASGVPSRFKGSGSGTQFTLTISGVQCDDAATYYCQGSYYNGAWYVAFGGGTELEIKRDPVAPSVLLFPPSKEELTTGTATIVCVANKFYPSDITVTWKVDGTTQQSGIENSKTPQSPEDNTYSLSSTLSLTSAQYNSHSVYTCEVVQGSASPIVQSFNRGDC

SEQ ID NO: 9 - protein, 5 aa, Artificial Sequence
  synthetic peptide
  MISC_FEATURE (1)..(5): X may be any amino acid, provided at least one of X1, X2, X4 or X5 is a D amino acid and/or a non-standard or non-natural amino acid
  MOD_RES (3)..(3): Amino acid has a Gal-Sial group
XXXXX

SEQ ID NO: 10 - protein, 20 aa, ARTIFICIAL
  synthetic peptide
  MISC_FEATURE (1)..(1): X is absent or Thr
  MISC_FEATURE (2)..(2): X is absent or Ala in D form
  MISC_FEATURE (3)..(3): X is absent or Norleucine
  MISC_FEATURE (4)..(4): X is absent or Glu
  MISC_FEATURE (5)..(5): X is absent or Ala in D form
  MISC_FEATURE (6)..(6): X is absent or Arg
  MISC_FEATURE (7)..(7): X is absent or selected from Glu, Arg, Ser, Norvaline, beta-Ala
  MISC_FEATURE (8)..(8): X is absent or selected from Ser in D form, Ala in D form, Phosphoserine, 1-aminocyclohexane-carboxylic acid
  MISC_FEATURE (9)..(9): X is absent or selected from Norvaline, 2'-(aminomethyl)biphenyl-2-carboxylic acid , Ala in D form, beta-Ala, Ornithine
  MISC_FEATURE (10)..(10): X is selected from 1-aminocyclohexane-carboxylic acid , Ser, Ile, Ala in D form, Ser in D form
  MISC_FEATURE (11)..(11): X is selected from Ala in D form, Pro, Ornithine, Norleucine
  MISC_FEATURE (12)..(12): X is selected from Ser, Thr, Tyr, hydroxylysine, hydroxyproline, Asn, Arg or Phosphoserine; and has a Gal-Sial group
  MISC_FEATURE (13)..(13): X is selected from Ala in D form, 2'-(aminomethyl)biphenyl-2-carboxylic acid, beta-Ala
  MISC_FEATURE (14)..(14): X is selected from Arg, Asp in D form, Norleucine, Ornithine, Norvaline
  MISC_FEATURE (15)..(15): X is absent or selected from Phe, 2'-(aminomethyl)biphenyl-2-carboxylic acid, Ser, Glu, Ala in D form, Ser in D form
  MISC_FEATURE (16)..(16): X is absent or selected from Ser in D form, Glu
  MISC_FEATURE (17)..(17): X is absent or selected from Val, Ser, Thr
  MISC_FEATURE (18)..(18): X is absent or cyclohexylalanine
  MISC_FEATURE (19)..(19): X is absent or Ser in D form
  MISC_FEATURE (20)..(20): X is absent or Val
XXXXXXXXXXXXXXXXXXXX

SEQ ID NO: 11 - protein, 5 aa, artificial
  synthetic peptide
  MOD_RES (1)..(1): X is 1-aminocyclohexane-carboxylic acid
  MOD_RES (2)..(4): Each alanine is in the D form
  MOD_RES (3)..(3): Serine has a Gal-Sial group
XASAR

SEQ ID NO: 12 - protein, 11 aa, artificial sequence
  synthetic peptide
  MISC_FEATURE (2)..(2): Serine is in the D form
  MISC_FEATURE (3)..(3): X is norvaline
  MISC_FEATURE (4)..(4): X is 1-aminocyclohexane-carboxylic acid
  MISC_FEATURE (5)..(7): Each alanine is in the D form
  MOD_RES (5)..(5): Serine has a Gal-Sial group
  MISC_FEATURE (10)..(10): Serine is in the D form
ESXXASARFSV

SEQ ID NO: 13 - protein, 9 aa, artificial sequence
  synthetic peptide
  MISC_FEATURE (2)..(7): Each alanine is in the D form
  MISC_FEATURE (3)..(3): X is 2'-(aminomethyl)biphenyl-2-carboxylic acid
  MOD_RES (6)..(6): Serine has a Gal-Sial group
  MISC_FEATURE (8)..(8): Asp is in the D form
RAXSPSADS

SEQ ID NO: 14 - protein, 9 aa, artificial sequence
  synthetic peptide
  MOD_RES (2)..(2): Serine is phosphoserine
  MOD_RES (3)..(7): Each alanine is in the D form
  MISC_FEATURE (5)..(5): X is Ornithine
  MOD_RES (6)..(6): Serine has a Gal-Sial group
  MISC_FEATURE (8)..(8): X is norleucine
SSAIXSAXE

SEQ ID NO: 15 - protein, 13 aa, artificial sequence
  synthetic peptide
  MISC_FEATURE (1)..(1): Alanine is in the D form
  MISC_FEATURE (3)..(3): x is norvaline
  MISC_FEATURE (4)..(4): Serine is in the D form
  MISC_FEATURE (5)..(5): x is beta-alanine
  MISC_FEATURE (6)..(11): Each alanine is in the D form
  MISC_FEATURE (7)..(7): x is norleucine
  MOD_RES (8)..(8): Serine has a Gal-Sial group
  MISC_FEATURE (9)..(9): X is 2'-(aminomethyl)biphenyl-2-carboxylic acid
  MISC_FEATURE (10)..(10): X is Ornithine
ARXSXAXSXXAES

SEQ ID NO: 16 - protein, 20 aa, artificial sequence
  synthetic peptide
  MISC_FEATURE (2)..(5): Each Alanine is in the D form
  MISC_FEATURE (3)..(3): X is norleucine
  MISC_FEATURE (7)..(7): X is beta-alanine
  MISC_FEATURE (8)..(8): X is 1-aminocyclohexane-carboxylic acid
  MISC_FEATURE (9)..(9): X is Ornithine
  MISC_FEATURE (10)..(10): Serine is in the D form
  MOD_RES (12)..(12): Serine has a Gal-Sial group
  MISC_FEATURE (13)..(13): X is beta-alanine
  MISC_FEATURE (14)..(14): X is norvaline
  MISC_FEATURE (15)..(19): Serine is in the D form
  MISC_FEATURE (18)..(18): X is cyclohexylalanine
TAXEARXXXSPSXXSETXSV

SEQ ID NO: 17 - protein, 5 aa, artificial sequence
  synthetic peptide
  MISC_FEATURE (1)..(1): X may be any amino acid provided that at least one of X1, X2, X4 and X5 is a D-amino acid and/or a non-standard amino acid or a non-natural amino acid.
  MISC_FEATURE (2)..(2): X may be any amino acid provided that at least one of X1, X2, X4 and X5 is a D-amino acid and/or a non-standard amino acid or a non-natural amino acid.
  MISC_FEATURE (3)..(3): X is an amino acid comprising a Gal-Sial group and is selected from Ser, Thr, Tyr, hydroxylysine, hydroxyproline, Asn, Arg or phosphoserine
  MISC_FEATURE (4)..(4): X may be any amino acid provided that at least one of X1, X2, X4 and X5 is a D-amino acid and/or a non-standard amino acid or a non-natural amino acid.
  MISC_FEATURE (5)..(5): X may be any amino acid provided that at least one of X1, X2, X4 and X5 is a D-amino acid and/or a non-standard amino acid or a non-natural amino acid.
XXXXX